European Patent Specification EP 4 436 611 B1, published March 18, 2026. Title: Complexes comprising a shielding component. Applicant: Polypeptide Therapeutic Solutions S.L. The sequence listing filed with the application follows.

SEQUENCE LISTING (1 sequence)

SEQ ID NO: 1 - DNA, 5580 bp, synthetic construct
  misc_feature 1..5580: note = clDNA
  source 1..5580: mol_type = other DNA
gcgtataatggactattgtgtgctgataggtctcgccctgatttaaatcgtcgaccgttacataacttacggtaaatggcccgcctggctgaccgcccaacgacccccgcccattgacgtcaataatgacgtatgttcccatagtaacgccaatagggactttccattgacgtcaatgggtggagtatttacggtaaactgcccacttggcagtacatcaagtgtatcatatgccaagtacgccccctattgacgtcaatgacggtaaatggcccgcctggcattatgcccagtacatgaccttatgggactttcctacttggcagtacatctacgtattagtcatcgctattaccatggtgatgcggttttggcagtacatcaatgggcgtggatagcggtttgactcacggggatttccaagtctccaccccattgacgtcaatgggagtttgttttggcaccaaaatcaacgggactttccaaaatgtcgtaacaactccgccccattgacgcaaatgggcggtaggcgtgtacggtgggaggtctatataagcagagctcgtttagtgaaccgtcagatcgcctggagacgccatccacgctgttttgacctccatagaagacaccgggaccgatccagcctccggactctagaggatccggtactcgaggaactgaaaaaccagaaagttaactggtaagtttagtctttttgtcttttatttcaggtcccggatccggtggtggtgcaaatcaaagaactgctcctcagtggatgttgcctttacttctaggcctgtacggaagtgttacttctgctctaaaagctgcggaattgtacccgcggcccgggatccaccggtcgccaccatggaagacgccaaaaacataaagaaaggcccggcgccattctatcctctagaggatggaaccgctggagagcaactgcataaggctatgaagagatacgccctggttcctggaacaattgcttttacagatgcacatatcgaggtgaacatcacgtacgcggaatacttcgaaatgtccgttcggttggcagaagctatgaaacgatatgggctgaatacaaatcacagaatcgtcgtatgcagtgaaaactctcttcaattctttatgccggtgttgggcgcgttatttatcggagttgcagttgcgcccgcgaacgacatttataatgaacgtgaattgctcaacagtatgaacatttcgcagcctaccgtagtgtttgtttccaaaaaggggttgcaaaaaattttgaacgtgcaaaaaaaattaccaataatccagaaaattattatcatggattctaaaacggattaccagggatttcagtcgatgtacacgttcgtcacatctcatctacctcccggttttaatgaatacgattttgtaccagagtcctttgatcgtgacaaaacaattgcactgataatgaattcctctggatctactgggttacctaagggtgtggcccttccgcatagaactgcctgcgtcagattctcgcatgccagagatcctatttttggcaatcaaatcattccggatactgcgattttaagtgttgttccattccatcacggttttggaatgtttactacactcggatatttgatatgtggatttcgagtcgtcttaatgtatagatttgaagaagagctgtttttacgatcccttcaggattacaaaattcaaagtgcgttgctagtaccaaccctattttcattcttcgccaaaagcactctgattgacaaatacgatttatctaatttacacgaaattgcttctgggggcgcacctctttcgaaagaagtcggggaagcggttgcaaaacgcttccatcttccagggatacgacaaggatatgggctcactgagactacatcagctattctgattacacccgagggggatgataaaccgggcgcggtcggtaaagttgttccattttttgaagcgaaggttgtggatctggataccgggaaaacgctgggcgttaatcagagaggcgaattatgtgtcagaggacctatgattatgtccggttatgtaaacaatccggaagcgaccaacgccttgattgacaaggatggatggctacattctggagacatagcttactgggacgaagacgaacacttcttcatagttgaccgcttgaagtctttaattaaatacaaaggatatcaggtggcccccgctgaattggaatcgatattgttacaacaccccaacatcttcgacgcgggcgtggcaggtcttcccgacgatgacgccggtgaacttcccgccgccgttgttgttttggagcacggaaagacgatgacggaaaaagagatcgtggattacgtcgccagtcaagtaacaaccgcgaaaaagttgcgcggaggagttgtgtttgtggacgaagtaccgaaaggtcttaccggaaaactcgacgcaagaaaaatcagagagatcctcataaaggccaagaagggcggaaagtccaaattgtaaagcggccgcggggatccagacatgataagatacattgatgagtttggacaaaccacaactagaatgcagtgaaaaaaatgctttatttgtgaaatttgtgatgctattgctttatttgtaaccattataagctgcaataaacaagttaacaacaacaattgcattcattttatgtttcaggttcagggggaggtgtgggaggttttttagtcgaccatttaaatcggtctcgagggtatcagcacacaattgcccattatacgcgcgtataatgggcaattgtgtgctgataccctcgagaccgatttaaatggtcgactaaaaaacctcccacacctccccctgaacctgaaacataaaatgaatgcaattgttgttgttaacttgtttattgcagcttataatggttacaaataaagcaatagcatcacaaatttcacaaataaagcatttttttcactgcattctagttgtggtttgtccaaactcatcaatgtatcttatcatgtctggatccccgcggccgctttacaatttggactttccgcccttcttggcctttatgaggatctctctgatttttcttgcgtcgagttttccggtaagacctttcggtacttcgtccacaaacacaactcctccgcgcaactttttcgcggttgttacttgactggcgacgtaatccacgatctctttttccgtcatcgtctttccgtgctccaaaacaacaacggcggcgggaagttcaccggcgtcatcgtcgggaagacctgccacgcccgcgtcgaagatgttggggtgttgtaacaatatcgattccaattcagcgggggccacctgatatcctttgtatttaattaaagacttcaagcggtcaactatgaagaagtgttcgtcttcgtcccagtaagctatgtctccagaatgtagccatccatccttgtcaatcaaggcgttggtcgcttccggattgtttacataaccggacataatcataggtcctctgacacataattcgcctctctgattaacgcccagcgttttcccggtatccagatccacaaccttcgcttcaaaaaatggaacaactttaccgaccgcgcccggtttatcatccccctcgggtgtaatcagaatagctgatgtagtctcagtgagcccatatccttgtcgtatccctggaagatggaagcgttttgcaaccgcttccccgacttctttcgaaagaggtgcgcccccagaagcaatttcgtgtaaattagataaatcgtatttgtcaatcagagtgcttttggcgaagaatgaaaatagggttggtactagcaacgcactttgaattttgtaatcctgaagggatcgtaaaaacagctcttcttcaaatctatacattaagacgactcgaaatccacatatcaaatatccgagtgtagtaaacattccaaaaccgtgatggaatggaacaacacttaaaatcgcagtatccggaatgatttgattgccaaaaataggatctctggcatgcgagaatctgacgcaggcagttctatgcggaagggccacacccttaggtaacccagtagatccagaggaattcattatcagtgcaattgttttgtcacgatcaaaggactctggtacaaaatcgtattcattaaaaccgggaggtagatgagatgtgacgaacgtgtacatcgactgaaatccctggtaatccgttttagaatccatgataataattttctggattattggtaattttttttgcacgttcaaaattttttgcaacccctttttggaaacaaacactacggtaggctgcgaaatgttcatactgttgagcaattcacgttcattataaatgtcgttcgcgggcgcaactgcaactccgataaataacgcgcccaacaccggcataaagaattgaagagagttttcactgcatacgacgattctgtgatttgtattcagcccatatcgtttcatagcttctgccaaccgaacggacatttcgaagtattccgcgtacgtgatgttcacctcgatatgtgcatctgtaaaagcaattgttccaggaaccagggcgtatctcttcatagccttatgcagttgctctccagcggttccatcctctagaggatagaatggcgccgggcctttctttatgtttttggcgtcttccatggtggcgaccggtggatcccgggccgcgggtacaattccgcagcttttagagcagaagtaacacttccgtacaggcctagaagtaaaggcaacatccactgaggagcagttctttgatttgcaccaccaccggatccgggacctgaaataaaagacaaaaagactaaacttaccagttaactttctggtttttcagttcctcgagtaccggatcctctagagtccggaggctggatcggtcccggtgtcttctatggaggtcaaaacagcgtggatggcgtctccaggcgatctgacggttcactaaacgagctctgcttatatagacctcccaccgtacacgcctaccgcccatttgcgtcaatggggcggagttgttacgacattttggaaagtcccgttgattttggtgccaaaacaaactcccattgacgtcaatggggtggagacttggaaatccccgtgagtcaaaccgctatccacgcccattgatgtactgccaaaaccgcatcaccatggtaatagcgatgactaatacgtagatgtactgccaagtaggaaagtcccataaggtcatgtactgggcataatgccaggcgggccatttaccgtcattgacgtcaatagggggcgtacttggcatatgatacacttgatgtactgccaagtgggcagtttaccgtaaatactccacccattgacgtcaatggaaagtccctattggcgttactatgggaacatacgtcattattgacgtcaatgggcgggggtcgttgggcggtcagccaggcgggccatttaccgtaagttatgtaacggtcgacgatttaaatcagggcgagacctatcagcacacaatagtccattatacgc